European Patent Application EP 4 495 141 A2, published January 22, 2025. Title: Chimeric Antigen Receptor. Applicant: Noile-Immune Biotech, Inc. The sequence listing filed with the application follows.

SEQUENCE LISTING (68 sequences)

SEQ ID NO: 1 - DNA, 360 bp, synthetic construct
  misc_feature 1..360: note = VH region of anti-GM2 antibody for VL15VH
  source 1..360: mol_type = other DNA
gaagtgcagctggtgcagtccggagccgaggtgaaaaagcctggcgcctccgtcaaggtgagctgcaaggccagcggctatacattcaccgactataacatggactgggtgaagcagagccccggccagggactggagtggatgggctacatctaccccaataacggcggcaccggctacaaccagaagttcaagtccaaggtgaccatcaccgtggacaccagcaccagcaccgcctacatggaactgcacagcctcagaagcgaagacaccgctgtgtactactgcgccacctacggccactactacggctacatgttcgcctactggggacagggcaccctggtgaccgtcagcagc

SEQ ID NO: 2 - protein, 120 aa, synthetic construct
  REGION 1..120: note = VH region of anti-GM2 antibody
EVQLVQSGAEVKKPGASVKVSCKASGYTFTDYNMDWVKQSPGQGLEWMGYIYPNNGGTGYNQKFKSKVTITVDTSTSTAYMELHSLRSEDTAVYYCATYGHYYGYMFAYWGQGTLVTVSS

SEQ ID NO: 3 - DNA, 318 bp, synthetic construct
  misc_feature 1..318: note = VL region of anti-GM2 antibody for VL15VH
  source 1..318: mol_type = other DNA
gacatccagctgacccagtcccctagcagcctgtccgctagccccggagacagagtgaccatcacctgttccgccagctccagcgtgagctacatgcactggttccagcagaagcccggcaaggcccccaagctgtggatctacagcaccagcaacctggcttccggcgtgcctgccagattttccggctccggcagcggcacaagctactccctgaccatcagcagactgcagcccgaagacatcgccacctactactgtcagcagaggagcagctacccctacaccttcggcggcggcaccaaggtggagatcaag

SEQ ID NO: 4 - protein, 106 aa, synthetic construct
  REGION 1..106: note = VL region of anti-GM2 antibody
DIQLTQSPSSLSASPGDRVTITCSASSSVSYMHWFQQKPGKAPKLWIYSTSNLASGVPARFSGSGSGTSYSLTISRLQPEDIATYYCQQRSSYPYTFGGGTKVEIK

SEQ ID NO: 5 - DNA, 45 bp, synthetic construct
  misc_feature 1..45: note = Linker 15 for VL15VH
  source 1..45: mol_type = other DNA
ggcggcggcggaagcggaggcggcggcagcggcggaggcggaagc

SEQ ID NO: 6 - protein, 15 aa, synthetic construct
  REGION 1..15: note = Linker 15
GGGGSGGGGSGGGGS

SEQ ID NO: 7 - DNA, 75 bp, synthetic construct
  misc_feature 1..75: note = Linker 25 for VL25VH
  source 1..75: mol_type = other DNA
agctccgctgacgacgctaagaaggacgctgccaagaaggacgacgccaagaaggatgacgccaaaaaagacggc

SEQ ID NO: 8 - protein, 25 aa, synthetic construct
  REGION 1..25: note = Linker 25
SSADDAKKDAAKKDDAKKDDAKKDG

SEQ ID NO: 9 - DNA, 723 bp, synthetic construct
  misc_feature 1..723: note = anti-GM2scFv (VL15VH)
  source 1..723: mol_type = other DNA
gacatccagctgacccagtcccctagcagcctgtccgctagccccggagacagagtgaccatcacctgttccgccagctccagcgtgagctacatgcactggttccagcagaagcccggcaaggcccccaagctgtggatctacagcaccagcaacctggcttccggcgtgcctgccagattttccggctccggcagcggcacaagctactccctgaccatcagcagactgcagcccgaagacatcgccacctactactgtcagcagaggagcagctacccctacaccttcggcggcggcaccaaggtggagatcaagggcggcggcggaagcggaggcggcggcagcggcggaggcggaagcgaagtgcagctggtgcagtccggagccgaggtgaaaaagcctggcgcctccgtcaaggtgagctgcaaggccagcggctatacattcaccgactataacatggactgggtgaagcagagccccggccagggactggagtggatgggctacatctaccccaataacggcggcaccggctacaaccagaagttcaagtccaaggtgaccatcaccgtggacaccagcaccagcaccgcctacatggaactgcacagcctcagaagcgaagacaccgctgtgtactactgcgccacctacggccactactacggctacatgttcgcctactggggacagggcaccctggtgaccgtcagcagc

SEQ ID NO: 10 - protein, 241 aa, synthetic construct
  REGION 1..241: note = anti-GM2scFv (VL15VH)
DIQLTQSPSSLSASPGDRVTITCSASSSVSYMHWFQQKPGKAPKLWIYSTSNLASGVPARFSGSGSGTSYSLTISRLQPEDIATYYCQQRSSYPYTFGGGTKVEIKGGGGSGGGGSGGGGSEVQLVQSGAEVKKPGASVKVSCKASGYTFTDYNMDWVKQSPGQGLEWMGYIYPNNGGTGYNQKFKSKVTITVDTSTSTAYMELHSLRSEDTAVYYCATYGHYYGYMFAYWGQGTLVTVSS

SEQ ID NO: 11 - DNA, 753 bp, synthetic construct
  misc_feature 1..753: note = anti-GM2scFv (VL25VH)
  source 1..753: mol_type = other DNA
gatatccaactgacccagtccccttccagcctgagcgcttcccccggagacagggtgacaattacctgcagcgccagctcctccgtgagctacatgcactggttccagcagaagcccggcaaggcccccaagctgtggatctactccacaagcaacctggcctccggcgtgcctgccagatttagcggaagcggcagcggcacatcctacagcctgaccatctccaggctgcagcccgaggacatcgccacatactactgccagcagaggtccagctacccttacacattcggaggcggcaccaaggtggagatcaagagctccgctgacgacgctaagaaggacgctgccaagaaggacgacgccaagaaggatgacgccaaaaaagacggcgaagtccagctggtgcagagcggcgctgaggtgaagaagcctggcgccagcgtcaaggtgagctgtaaggcctccggctacaccttcaccgactacaacatggattgggtgaagcagagccccggacagggcctggagtggatgggctacatctaccccaacaacggcggcaccggctacaaccagaaattcaagtccaaggtgaccatcaccgtggacaccagcacatccaccgcctacatggaactgcacagcctgaggtccgaggacacagccgtgtactactgcgctacctacggccactactacggctacatgttcgcttactggggacagggcaccctggtgaccgtgagctcc

SEQ ID NO: 12 - protein, 251 aa, synthetic construct
  REGION 1..251: note = anti-GM2scFv (VL25VH)
DIQLTQSPSSLSASPGDRVTITCSASSSVSYMHWFQQKPGKAPKLWIYSTSNLASGVPARFSGSGSGTSYSLTISRLQPEDIATYYCQQRSSYPYTFGGGTKVEIKSSADDAKKDAAKKDDAKKDDAKKDGEVQLVQSGAEVKKPGASVKVSCKASGYTFTDYNMDWVKQSPGQGLEWMGYIYPNNGGTGYNQKFKSKVTITVDTSTSTAYMELHSLRSEDTAVYYCATYGHYYGYMFAYWGQGTLVTVSS

SEQ ID NO: 13 - DNA, 723 bp, synthetic construct
  misc_feature 1..723: note = anti-GM2scFv (VH15VL)
  source 1..723: mol_type = other DNA
gaggtgcagctggtgcagtccggagccgaggtgaagaagcctggcgccagcgtgaaggtgagctgtaaggcctccggctacaccttcaccgactacaacatggactgggtcaagcagagccctggccagggcctggagtggatgggctatatctaccccaacaacggcggcaccggctacaaccagaagttcaagagcaaggtcaccatcaccgtggacacctccacctccacagcctacatggagctgcacagcctgaggagcgaggataccgccgtgtactactgcgctacctacggccattactacggatacatgttcgcctactggggccagggaaccctggtcaccgtgtcctccggaggaggaggaagcggaggcggcggctccggcggaggcggatccgacatccagctgacacaatcccccagcagcctgagcgctagccccggcgatagggtgacaattacctgcagcgcctccagctccgtgtcctacatgcactggtttcagcaaaagcccggcaaggcccctaagctgtggatctacagcaccagcaacctggccagcggagtgcctgccagatttagcggcagcggcagcggcaccagctacagcctgaccatcagcagactgcagcccgaggatatcgccacctactactgccagcagaggagctcctacccctacacattcggcggcggaaccaaggtggagatcaag

SEQ ID NO: 14 - protein, 241 aa, synthetic construct
  REGION 1..241: note = anti-GM2scFv (VH15VL)
EVQLVQSGAEVKKPGASVKVSCKASGYTFTDYNMDWVKQSPGQGLEWMGYIYPNNGGTGYNQKFKSKVTITVDTSTSTAYMELHSLRSEDTAVYYCATYGHYYGYMFAYWGQGTLVTVSSGGGGSGGGGSGGGGSDIQLTQSPSSLSASPGDRVTITCSASSSVSYMHWFQQKPGKAPKLWIYSTSNLASGVPARFSGSGSGTSYSLTISRLQPEDIATYYCQQRSSYPYTFGGGTKVEIK

SEQ ID NO: 15 - DNA, 753 bp, synthetic construct
  misc_feature 1..753: note = anti-GM2scFv (VH25VL)
  source 1..753: mol_type = other DNA
gaagtgcagctggtgcagtccggagctgaggtgaagaagcccggcgccagcgtgaaggtcagctgcaaagccagcggctataccttcaccgactacaacatggactgggtgaagcagagccccggccaaggcctcgagtggatgggatacatctaccccaacaacggcggcaccggctacaaccagaagttcaagagcaaggtgaccatcaccgtggacacatccacaagcaccgcctatatggagctccacagcctgaggagcgaggacaccgccgtgtactactgcgccacctacggccactactacggctatatgttcgcctactggggccagggcaccctggtgacagtgtcctcctccagcgccgatgatgccaagaaggatgccgccaaaaaggacgacgctaagaaggatgacgccaagaaggacggcgatatccagctgacacagagccctagctccctgagcgctagccctggcgacagagtgaccatcacctgcagcgccagctccagcgtgagctacatgcactggttccagcagaaacccggcaaggcccccaagctgtggatctacagcaccagcaatctggctagcggcgtgcctgccaggtttagcggatccggcagcggcacctcctactccctgacaatctccagactgcagcccgaggacatcgccacctactactgccaacagaggtcctcctacccctacaccttcggcggcggcaccaaagtggagatcaag

SEQ ID NO: 16 - protein, 251 aa, synthetic construct
  REGION 1..251: note = anti-GM2scFv (VH25VL)
EVQLVQSGAEVKKPGASVKVSCKASGYTFTDYNMDWVKQSPGQGLEWMGYIYPNNGGTGYNQKFKSKVTITVDTSTSTAYMELHSLRSEDTAVYYCATYGHYYGYMFAYWGQGTLVTVSSSSADDAKKDAAKKDDAKKDDAKKDGDIQLTQSPSSLSASPGDRVTITCSASSSVSYMHWFQQKPGKAPKLWIYSTSNLASGVPARFSGSGSGTSYSLTISRLQPEDIATYYCQQRSSYPYTFGGGTKVEIK

SEQ ID NO: 17 - DNA, 165 bp, Homo sapiens
  source 1..165: mol_type = other DNA
ttcgtgccggtcttcctgccagcgaagcccaccacgacgccagcgccgcgaccaccaacaccggcgcccaccatcgcgtcgcagcccctgtccctgcgcccagaggcgtgccggccagcggcggggggcgcagtgcacacgagggggctggacttcgcctgtgat

SEQ ID NO: 18 - protein, 55 aa, Homo sapiens
FVPVFLPAKPTTTPAPRPPTPAPTIASQPLSLRPEACRPAAGGAVHTRGLDFACD

SEQ ID NO: 19 - DNA, 63 bp, Homo sapiens
  source 1..63: mol_type = other DNA
atctacatctgggcgcccttggccgggacttgtggggtccttctcctgtcactggttatcacc

SEQ ID NO: 20 - protein, 21 aa, Homo sapiens
IYIWAPLAGTCGVLLLSLVIT

SEQ ID NO: 21 - DNA, 21 bp, Homo sapiens
  source 1..21: mol_type = other DNA
ctttactgcaaccacaggaac

SEQ ID NO: 22 - protein, 7 aa, Homo sapiens
LYCNHRN

SEQ ID NO: 23 - DNA, 123 bp, Homo sapiens
  source 1..123: mol_type = other DNA
aggagtaagaggagcaggctcctgcacagtgactacatgaacatgactccccgccgccccgggcccacccgcaagcattaccagccctatgccccaccacgcgacttcgcagcctatcgctcc

SEQ ID NO: 24 - protein, 41 aa, Homo sapiens
RSKRSRLLHSDYMNMTPRRPGPTRKHYQPYAPPRDFAAYRS

SEQ ID NO: 25 - DNA, 138 bp, Homo sapiens
  source 1..138: mol_type = other DNA
cgtttctctgttgttaaacggggcagaaagaagctcctgtatatattcaaacaaccatttatgagaccagtacaaactactcaagaggaagatggctgtagctgccgatttccagaagaagaagaaggaggatgtgaa

SEQ ID NO: 26 - protein, 46 aa, Homo sapiens
RFSVVKRGRKKLLYIFKQPFMRPVQTTQEEDGCSCRFPEEEEGGCE

SEQ ID NO: 27 - DNA, 339 bp, Homo sapiens
  source 1..339: mol_type = other DNA
ctgagagtgaagttcagcaggagcgcagacgcccccgcgtaccagcagggccagaaccagctctataacgagctcaatctaggacgaagagaggagtacgatgttttggacaagagacgtggccgggaccctgagatggggggaaagccgagaaggaagaaccctcaggaaggcctgtacaatgaactgcagaaagataagatggcggaggcctacagtgagattgggatgaaaggcgagcgccggaggggcaaggggcacgatggcctttaccagggtctcagtacagccaccaaggacacctacgacgcccttcacatgcaggccctgccccctcgc

SEQ ID NO: 28 - protein, 113 aa, Homo sapiens
LRVKFSRSADAPAYQQGQNQLYNELNLGRREEYDVLDKRRGRDPEMGGKPRRKNPQEGLYNELQKDKMAEAYSEIGMKGERRRGKGHDGLYQGLSTATKDTYDALHMQALPPR

SEQ ID NO: 29 - DNA, 849 bp, synthetic construct
  misc_feature 1..849: note = CD8 (hinge)_CD8 (transmembrane)_CD28 (signaling)_4-1BB (signaling)_CD3z (signaling)
  source 1..849: mol_type = other DNA
ttcgtgccggtcttcctgccagcgaagcccaccacgacgccagcgccgcgaccaccaacaccggcgcccaccatcgcgtcgcagcccctgtccctgcgcccagaggcgtgccggccagcggcggggggcgcagtgcacacgagggggctggacttcgcctgtgatatctacatctgggcgcccttggccgggacttgtggggtccttctcctgtcactggttatcaccctttactgcaaccacaggaacaggagtaagaggagcaggctcctgcacagtgactacatgaacatgactccccgccgccccgggcccacccgcaagcattaccagccctatgccccaccacgcgacttcgcagcctatcgctcccgtttctctgttgttaaacggggcagaaagaagctcctgtatatattcaaacaaccatttatgagaccagtacaaactactcaagaggaagatggctgtagctgccgatttccagaagaagaagaaggaggatgtgaactgagagtgaagttcagcaggagcgcagacgcccccgcgtaccagcagggccagaaccagctctataacgagctcaatctaggacgaagagaggagtacgatgttttggacaagagacgtggccgggaccctgagatggggggaaagccgagaaggaagaaccctcaggaaggcctgtacaatgaactgcagaaagataagatggcggaggcctacagtgagattgggatgaaaggcgagcgccggaggggcaaggggcacgatggcctttaccagggtctcagtacagccaccaaggacacctacgacgcccttcacatgcaggccctgccccctcgc

SEQ ID NO: 30 - protein, 283 aa, synthetic construct
  REGION 1..283: note = CD8 (hinge)_CD8 (transmembrane)_CD28 (signaling)_4-1BB (signaling)_CD3z (signaling)
FVPVFLPAKPTTTPAPRPPTPAPTIASQPLSLRPEACRPAAGGAVHTRGLDFACDIYIWAPLAGTCGVLLLSLVITLYCNHRNRSKRSRLLHSDYMNMTPRRPGPTRKHYQPYAPPRDFAAYRSRFSVVKRGRKKLLYIFKQPFMRPVQTTQEEDGCSCRFPEEEEGGCELRVKFSRSADAPAYQQGQNQLYNELNLGRREEYDVLDKRRGRDPEMGGKPRRKNPQEGLYNELQKDKMAEAYSEIGMKGERRRGKGHDGLYQGLSTATKDTYDALHMQALPPR

SEQ ID NO: 31 - DNA, 86 bp, synthetic construct
  misc_feature 1..86: note = EcoRI_F2A-NsiI
  source 1..86: mol_type = other DNA
gaattcggaagcggagtgaaacagactttgaattttgaccttctcaagttggcgggagacgtggagtccaaccctggaccatgcat

SEQ ID NO: 32 - protein, 28 aa, synthetic construct
  REGION 1..28: note = EcoRI_F2A-NsiI
EFGSGVKQTLNFDLLKLAGDVESNPGPC

SEQ ID NO: 33 - DNA, 909 bp, synthetic construct
  misc_feature 1..909: note = IL7_F2A_CCL19_SalI
  source 1..909: mol_type = other DNA
atgttccatgtttcttttaggtatatctttggacttcctcccctgatccttgttctgttgccagtagcatcatctgattgtgatattgaaggtaaagatggcaaacaatatgagagtgttctaatggtcagcatcgatcaattattggacagcatgaaagaaattggtagcaattgcctgaataatgaatttaacttttttaaaagacatatctgtgatgctaataaggaaggtatgtttttattccgtgctgctcgcaagttgaggcaatttcttaaaatgaatagcactggtgattttgatctccacttattaaaagtttcagaaggcacaacaatactgttgaactgcactggccaggttaaaggaagaaaaccagctgccctgggtgaagcccaaccaacaaagagtttggaagaaaataaatctttaaaggaacagaaaaaactgaatgacttgtgtttcctaaagagactattacaagagataaaaacttgttggaataaaattttgatgggcactaaagaacacggaagcggagtgaaacagactttgaattttgaccttctcaagttggcgggagacgtggagtccaaccctggacctatggccctgctactggccctcagcctgctggttctctggacttccccagccccaactctgagtggcaccaatgatgctgaagactgctgcctgtctgtgacccagaaacccatccctgggtacatcgtgaggaacttccactaccttctcatcaaggatggctgcagggtgcctgctgtagtgttcaccacactgaggggccgccagctctgtgcacccccagaccagccctgggtagaacgcatcatccagagactgcagaggacctcagccaagatgaagcgccgcagcagttaagtcgac

SEQ ID NO: 34 - protein, 300 aa, synthetic construct
  REGION 1..300: note = IL7_F2A_CCL19_SalI
MFHVSFRYIFGLPPLILVLLPVASSDCDIEGKDGKQYESVLMVSIDQLLDSMKEIGSNCLNNEFNFFKRHICDANKEGMFLFRAARKLRQFLKMNSTGDFDLHLLKVSEGTTILLNCTGQVKGRKPAALGEAQPTKSLEENKSLKEQKKLNDLCFLKRLLQEIKTCWNKILMGTKEHGSGVKQTLNFDLLKLAGDVESNPGPMALLLALSLLVLWTSPAPTLSGTNDAEDCCLSVTQKPIPGYIVRNFHYLLIKDGCRVPAVVFTTLRGRQLCAPPDQPWVERIIQRLQRTSAKMKRRSS

SEQ ID NO: 35 - DNA, 2112 bp, synthetic construct
  misc_feature 1..2112: note = IL7_F2A_CCL19_HSVtK_SalI
  source 1..2112: mol_type = other DNA
atgttccatgtgagcttcaggtacatcttcggactgcctcctctcatcctggtcctcctccccgtggccagctccgactgtgacatcgaaggaaaggatggcaagcagtacgaaagcgtgctgatggtgagcatcgatcagctcctggattccatgaaggaaatcggctccaactgcctcaacaatgagttcaacttttttaagaggcatatctgcgacgccaacaaggagggcatgtttctgttcagggccgccaggaagctgagacagttcctcaagatgaatagcaccggcgacttcgacctccatctgctgaaggtgtccgagggaaccaccatcctgctgaactgcaccggccaagtgaagggaagaaaacctgctgccctgggcgaggctcagcctaccaagagcctcgaggagaacaaaagcctgaaggagcagaagaagctgaacgacctgtgcttcctcaagaggctcctgcaggagattaagacctgttggaacaagatcctgatgggcacaaaggagcacggatccggcgtgaagcagaccctgaactttgacctgctcaaactggccggcgacgtcgagtccaatcctggacctatggctctgctgctcgccctgagcctgctcgtcctctggacctcccctgctcctaccctgagcggcaccaatgacgctgaagactgctgcctgtccgtgacccagaagcctatccccggatatatcgtgaggaattttcattacctcctgatcaaggacggctgtagagtgcccgccgtcgtgttcacaacactcagaggcaggcagctgtgtgctccccccgaccagccttgggtggagagaatcattcagagactgcaaaggacctccgctaagatgaagaggaggtccagcggcagcggagtgaagcagacactgaatttcgacctgctcaagctggccggcgatgtggagagcaaccctggacctatggcttcctaccccggacatcagcacgcttccgccttcgaccaggccgctagaagcagaggacactccaatagaaggacagccctgaggcctaggagacagcaggaggccaccgaggtgaggcccgagcagaaaatgcccaccctgctgagagtgtatattgatggaccccacggcatgggaaaaaccaccacaacccagctgctggtggctctgggaagcagggatgatattgtgtacgtccccgaacctatgacatattggagggtcctcggcgcctccgagaccatcgccaacatttacaccacccagcacaggctggatcagggagagatctccgccggcgatgctgccgtggtgatgaccagcgcccagatcactatgggtatgccttatgccgtgaccgacgctgtgctggctcctcacattggcggcgaagccggatcctcccatgctccccctcctgccctcacactgatctttgacagacatcctatcgccgctctgctgtgctaccccgccgctaggtacctgatgggcagcatgacccctcaggccgtgctggcttttgtggccctcattccccccacactgcctggcacaaatatcgtgctcggcgccctgcctgaggacaggcacatcgataggctggctaagagacagagacccggagagaggctggatctcgctatgctggccgccatcaggagggtgtacggcctgctggccaacaccgtgagatatctccagtgtggcggatcctggagggaagactggggccaactgagcggcacagctgtgcctcctcaaggcgctgagccccagagcaacgctggacccagacctcacatcggcgataccctgttcaccctgtttagagcccctgagctcctggcccctaacggcgacctgtacaatgtgttcgcttgggccctggatgtgctcgccaagagactcaggagcatgcacgtcttcattctggactacgaccagtcccccgctggctgcagagatgccctgctccagctgacctccggcatggtgcagacccacgtgaccacccctggaagcatccccacaatctgcgacctggccaggacctttgccagagaaatgggagaagccaactgagtcgac

SEQ ID NO: 36 - protein, 701 aa, synthetic construct
  REGION 1..701: note = IL7_F2A_CCL19_HSVtK_SalI
MFHVSFRYIFGLPPLILVLLPVASSDCDIEGKDGKQYESVLMVSIDQLLDSMKEIGSNCLNNEFNFFKRHICDANKEGMFLFRAARKLRQFLKMNSTGDFDLHLLKVSEGTTILLNCTGQVKGRKPAALGEAQPTKSLEENKSLKEQKKLNDLCFLKRLLQEIKTCWNKILMGTKEHGSGVKQTLNFDLLKLAGDVESNPGPMALLLALSLLVLWTSPAPTLSGTNDAEDCCLSVTQKPIPGYIVRNFHYLLIKDGCRVPAVVFTTLRGRQLCAPPDQPWVERIIQRLQRTSAKMKRRSSGSGVKQTLNFDLLKLAGDVESNPGPMASYPGHQHASAFDQAARSRGHSNRRTALRPRRQQEATEVRPEQKMPTLLRVYIDGPHGMGKTTTTQLLVALGSRDDIVYVPEPMTYWRVLGASETIANIYTTQHRLDQGEISAGDAAVVMTSAQITMGMPYAVTDAVLAPHIGGEAGSSHAPPPALTLIFDRHPIAALLCYPAARYLMGSMTPQAVLAFVALIPPTLPGTNIVLGALPEDRHIDRLAKRQRPGERLDLAMLAAIRRVYGLLANTVRYLQCGGSWREDWGQLSGTAVPPQGAEPQSNAGPRPHIGDTLFTLFRAPELLAPNGDLYNVFAWALDVLAKRLRSMHVFILDYDQSPAGCRDALLQLTSGMVQTHVTTPGSIPTICDLARTFAREMGEAN

SEQ ID NO: 37 - DNA, 1641 bp, synthetic construct
  misc_feature 1..1641: note = anti-hCD20 CAR
  source 1..1641: mol_type = other DNA
atggattggacctggaggatcctgtttctggtggctgccgccaccggagcccattcccagatcgtgctgagccagagccctgccattctgagcgccagccccggcgaaaaggtgaccatgacctgcagggccagcagcagcgtgtcctacatccactggttccagcagaagcccggctccagccccaaaccctggatctacgccaccagcaatctggccagcggcgtgcctgtgagattctccggcagcggcagcggcacaagctatagcctgaccatctccagagtggaggccgaggatgccgccacctactactgccagcagtggaccagcaacccccccacattcggaggcggcaccaagctggagatcaaaggcggaggcggcagcggcggaggcggcagcggaggcggaggaagccaagtgcagctgcagcagcctggagctgagctggtgaagcctggcgcctccgtcaagatgagctgcaaggccagcggctacacattcaccagctacaacatgcactgggtgaagcagacccccggaagaggcctggagtggatcggagccatctaccccggcaacggcgataccagctataaccagaagttcaagggcaaggccaccctcaccgccgacaagagcagcagcaccgcctacatgcagctgagcagcctgacctccgaggacagcgccgtgtactactgcgccaggtccacctactatggcggcgactggtacttcaacgtgtggggcgccggaacaaccgtgaccgtgagcgccgcggccgcattcgtgccggtcttcctgccagcgaagcccaccacgacgccagcgccgcgaccaccaacaccggcgcccaccatcgcgtcgcagcccctgtccctgcgcccagaggcgtgccggccagcggcggggggcgcagtgcacacgagggggctggacttcgcctgtgatatctacatctgggcgcccttggccgggacttgtggggtccttctcctgtcactggttatcaccctttactgcaaccacaggaacaggagtaagaggagcaggctcctgcacagtgactacatgaacatgactccccgccgccccgggcccacccgcaagcattaccagccctatgccccaccacgcgacttcgcagcctatcgctcccgtttctctgttgttaaacggggcagaaagaagctcctgtatatattcaaacaaccatttatgagaccagtacaaactactcaagaggaagatggctgtagctgccgatttccagaagaagaagaaggaggatgtgaactgagagtgaagttcagcaggagcgcagacgcccccgcgtaccagcagggccagaaccagctctataacgagctcaatctaggacgaagagaggagtacgatgttttggacaagagacgtggccgggaccctgagatggggggaaagccgagaaggaagaaccctcaggaaggcctgtacaatgaactgcagaaagataagatggcggaggcctacagtgagattgggatgaaaggcgagcgccggaggggcaaggggcacgatggcctttaccagggtctcagtacagccaccaaggacacctacgacgcccttcacatgcaggccctgccccctcgc

SEQ ID NO: 38 - protein, 547 aa, synthetic construct
  REGION 1..547: note = anti-hCD20 CAR
MDWTWRILFLVAAATGAHSQIVLSQSPAILSASPGEKVTMTCRASSSVSYIHWFQQKPGSSPKPWIYATSNLASGVPVRFSGSGSGTSYSLTISRVEAEDAATYYCQQWTSNPPTFGGGTKLEIKGGGGSGGGGSGGGGSQVQLQQPGAELVKPGASVKMSCKASGYTFTSYNMHWVKQTPGRGLEWIGAIYPGNGDTSYNQKFKGKATLTADKSSSTAYMQLSSLTSEDSAVYYCARSTYYGGDWYFNVWGAGTTVTVSAAAAFVPVFLPAKPTTTPAPRPPTPAPTIASQPLSLRPEACRPAAGGAVHTRGLDFACDIYIWAPLAGTCGVLLLSLVITLYCNHRNRSKRSRLLHSDYMNMTPRRPGPTRKHYQPYAPPRDFAAYRSRFSVVKRGRKKLLYIFKQPFMRPVQTTQEEDGCSCRFPEEEEGGCELRVKFSRSADAPAYQQGQNQLYNELNLGRREEYDVLDKRRGRDPEMGGKPRRKNPQEGLYNELQKDKMAEAYSEIGMKGERRRGKGHDGLYQGLSTATKDTYDALHMQALPPR

SEQ ID NO: 39 - DNA, 2625 bp, synthetic construct
  misc_feature 1..2625: note = anti-GM2 CAR (VL15VH)
  source 1..2625: mol_type = other DNA
atggattggacctggaggattctgttcctggtggctgctgccacaggcgcccattccgacatccagctgacccagtcccctagcagcctgtccgctagccccggagacagagtgaccatcacctgttccgccagctccagcgtgagctacatgcactggttccagcagaagcccggcaaggcccccaagctgtggatctacagcaccagcaacctggcttccggcgtgcctgccagattttccggctccggcagcggcacaagctactccctgaccatcagcagactgcagcccgaagacatcgccacctactactgtcagcagaggagcagctacccctacaccttcggcggcggcaccaaggtggagatcaagggcggcggcggaagcggaggcggcggcagcggcggaggcggaagcgaagtgcagctggtgcagtccggagccgaggtgaaaaagcctggcgcctccgtcaaggtgagctgcaaggccagcggctatacattcaccgactataacatggactgggtgaagcagagccccggccagggactggagtggatgggctacatctaccccaataacggcggcaccggctacaaccagaagttcaagtccaaggtgaccatcaccgtggacaccagcaccagcaccgcctacatggaactgcacagcctcagaagcgaagacaccgctgtgtactactgcgccacctacggccactactacggctacatgttcgcctactggggacagggcaccctggtgaccgtcagcagcgcggccgcattcgtgccggtcttcctgccagcgaagcccaccacgacgccagcgccgcgaccaccaacaccggcgcccaccatcgcgtcgcagcccctgtccctgcgcccagaggcgtgccggccagcggcggggggcgcagtgcacacgagggggctggacttcgcctgtgatatctacatctgggcgcccttggccgggacttgtggggtccttctcctgtcactggttatcaccctttactgcaaccacaggaacaggagtaagaggagcaggctcctgcacagtgactacatgaacatgactccccgccgccccgggcccacccgcaagcattaccagccctatgccccaccacgcgacttcgcagcctatcgctcccgtttctctgttgttaaacggggcagaaagaagctcctgtatatattcaaacaaccatttatgagaccagtacaaactactcaagaggaagatggctgtagctgccgatttccagaagaagaagaaggaggatgtgaactgagagtgaagttcagcaggagcgcagacgcccccgcgtaccagcagggccagaaccagctctataacgagctcaatctaggacgaagagaggagtacgatgttttggacaagagacgtggccgggaccctgagatggggggaaagccgagaaggaagaaccctcaggaaggcctgtacaatgaactgcagaaagataagatggcggaggcctacagtgagattgggatgaaaggcgagcgccggaggggcaaggggcacgatggcctttaccagggtctcagtacagccaccaaggacacctacgacgcccttcacatgcaggccctgccccctcgcgaattcggaagcggagtgaaacagactttgaattttgaccttctcaagttggcgggagacgtggagtccaaccctggaccatgcatgttccatgtttcttttaggtatatctttggacttcctcccctgatccttgttctgttgccagtagcatcatctgattgtgatattgaaggtaaagatggcaaacaatatgagagtgttctaatggtcagcatcgatcaattattggacagcatgaaagaaattggtagcaattgcctgaataatgaatttaacttttttaaaagacatatctgtgatgctaataaggaaggtatgtttttattccgtgctgctcgcaagttgaggcaatttcttaaaatgaatagcactggtgattttgatctccacttattaaaagtttcagaaggcacaacaatactgttgaactgcactggccaggttaaaggaagaaaaccagctgccctgggtgaagcccaaccaacaaagagtttggaagaaaataaatctttaaaggaacagaaaaaactgaatgacttgtgtttcctaaagagactattacaagagataaaaacttgttggaataaaattttgatgggcactaaagaacacggaagcggagtgaaacagactttgaattttgaccttctcaagttggcgggagacgtggagtccaaccctggacctatggccctgctactggccctcagcctgctggttctctggacttccccagccccaactctgagtggcaccaatgatgctgaagactgctgcctgtctgtgacccagaaacccatccctgggtacatcgtgaggaacttccactaccttctcatcaaggatggctgcagggtgcctgctgtagtgttcaccacactgaggggccgccagctctgtgcacccccagaccagccctgggtagaacgcatcatccagagactgcagaggacctcagccaagatgaagcgccgcagcagttaa

SEQ ID NO: 40 - protein, 874 aa, synthetic construct
  REGION 1..874: note = anti-GM2 CAR (VL15VH)
MDWTWRILFLVAAATGAHSDIQLTQSPSSLSASPGDRVTITCSASSSVSYMHWFQQKPGKAPKLWIYSTSNLASGVPARFSGSGSGTSYSLTISRLQPEDIATYYCQQRSSYPYTFGGGTKVEIKGGGGSGGGGSGGGGSEVQLVQSGAEVKKPGASVKVSCKASGYTFTDYNMDWVKQSPGQGLEWMGYIYPNNGGTGYNQKFKSKVTITVDTSTSTAYMELHSLRSEDTAVYYCATYGHYYGYMFAYWGQGTLVTVSSAAAFVPVFLPAKPTTTPAPRPPTPAPTIASQPLSLRPEACRPAAGGAVHTRGLDFACDIYIWAPLAGTCGVLLLSLVITLYCNHRNRSKRSRLLHSDYMNMTPRRPGPTRKHYQPYAPPRDFAAYRSRFSVVKRGRKKLLYIFKQPFMRPVQTTQEEDGCSCRFPEEEEGGCELRVKFSRSADAPAYQQGQNQLYNELNLGRREEYDVLDKRRGRDPEMGGKPRRKNPQEGLYNELQKDKMAEAYSEIGMKGERRRGKGHDGLYQGLSTATKDTYDALHMQALPPREFGSGVKQTLNFDLLKLAGDVESNPGPCMFHVSFRYIFGLPPLILVLLPVASSDCDIEGKDGKQYESVLMVSIDQLLDSMKEIGSNCLNNEFNFFKRHICDANKEGMFLFRAARKLRQFLKMNSTGDFDLHLLKVSEGTTILLNCTGQVKGRKPAALGEAQPTKSLEENKSLKEQKKLNDLCFLKRLLQEIKTCWNKILMGTKEHGSGVKQTLNFDLLKLAGDVESNPGPMALLLALSLLVLWTSPAPTLSGTNDAEDCCLSVTQKPIPGYIVRNFHYLLIKDGCRVPAVVFTTLRGRQLCAPPDQPWVERIIQRLQRTSAKMKRRSS

SEQ ID NO: 41 - DNA, 2655 bp, synthetic construct
  misc_feature 1..2655: note = anti-GM2 CAR (VL25VH)
  source 1..2655: mol_type = other DNA
atggactggacctggaggatcctctttctggtggccgccgctaccggcgctcacagcgatatccaactgacccagtccccttccagcctgagcgcttcccccggagacagggtgacaattacctgcagcgccagctcctccgtgagctacatgcactggttccagcagaagcccggcaaggcccccaagctgtggatctactccacaagcaacctggcctccggcgtgcctgccagatttagcggaagcggcagcggcacatcctacagcctgaccatctccaggctgcagcccgaggacatcgccacatactactgccagcagaggtccagctacccttacacattcggaggcggcaccaaggtggagatcaagagctccgctgacgacgctaagaaggacgctgccaagaaggacgacgccaagaaggatgacgccaaaaaagacggcgaagtccagctggtgcagagcggcgctgaggtgaagaagcctggcgccagcgtcaaggtgagctgtaaggcctccggctacaccttcaccgactacaacatggattgggtgaagcagagccccggacagggcctggagtggatgggctacatctaccccaacaacggcggcaccggctacaaccagaaattcaagtccaaggtgaccatcaccgtggacaccagcacatccaccgcctacatggaactgcacagcctgaggtccgaggacacagccgtgtactactgcgctacctacggccactactacggctacatgttcgcttactggggacagggcaccctggtgaccgtgagctccgcggccgcattcgtgccggtcttcctgccagcgaagcccaccacgacgccagcgccgcgaccaccaacaccggcgcccaccatcgcgtcgcagcccctgtccctgcgcccagaggcgtgccggccagcggcggggggcgcagtgcacacgagggggctggacttcgcctgtgatatctacatctgggcgcccttggccgggacttgtggggtccttctcctgtcactggttatcaccctttactgcaaccacaggaacaggagtaagaggagcaggctcctgcacagtgactacatgaacatgactccccgccgccccgggcccacccgcaagcattaccagccctatgccccaccacgcgacttcgcagcctatcgctcccgtttctctgttgttaaacggggcagaaagaagctcctgtatatattcaaacaaccatttatgagaccagtacaaactactcaagaggaagatggctgtagctgccgatttccagaagaagaagaaggaggatgtgaactgagagtgaagttcagcaggagcgcagacgcccccgcgtaccagcagggccagaaccagctctataacgagctcaatctaggacgaagagaggagtacgatgttttggacaagagacgtggccgggaccctgagatggggggaaagccgagaaggaagaaccctcaggaaggcctgtacaatgaactgcagaaagataagatggcggaggcctacagtgagattgggatgaaaggcgagcgccggaggggcaaggggcacgatggcctttaccagggtctcagtacagccaccaaggacacctacgacgcccttcacatgcaggccctgccccctcgcgaattcggaagcggagtgaaacagactttgaattttgaccttctcaagttggcgggagacgtggagtccaaccctggaccatgcatgttccatgtttcttttaggtatatctttggacttcctcccctgatccttgttctgttgccagtagcatcatctgattgtgatattgaaggtaaagatggcaaacaatatgagagtgttctaatggtcagcatcgatcaattattggacagcatgaaagaaattggtagcaattgcctgaataatgaatttaacttttttaaaagacatatctgtgatgctaataaggaaggtatgtttttattccgtgctgctcgcaagttgaggcaatttcttaaaatgaatagcactggtgattttgatctccacttattaaaagtttcagaaggcacaacaatactgttgaactgcactggccaggttaaaggaagaaaaccagctgccctgggtgaagcccaaccaacaaagagtttggaagaaaataaatctttaaaggaacagaaaaaactgaatgacttgtgtttcctaaagagactattacaagagataaaaacttgttggaataaaattttgatgggcactaaagaacacggaagcggagtgaaacagactttgaattttgaccttctcaagttggcgggagacgtggagtccaaccctggacctatggccctgctactggccctcagcctgctggttctctggacttccccagccccaactctgagtggcaccaatgatgctgaagactgctgcctgtctgtgacccagaaacccatccctgggtacatcgtgaggaacttccactaccttctcatcaaggatggctgcagggtgcctgctgtagtgttcaccacactgaggggccgccagctctgtgcacccccagaccagccctgggtagaacgcatcatccagagactgcagaggacctcagccaagatgaagcgccgcagcagttaa

SEQ ID NO: 42 - protein, 884 aa, synthetic construct
  REGION 1..884: note = anti-GM2 CAR (VL25VH)
MDWTWRILFLVAAATGAHSDIQLTQSPSSLSASPGDRVTITCSASSSVSYMHWFQQKPGKAPKLWIYSTSNLASGVPARFSGSGSGTSYSLTISRLQPEDIATYYCQQRSSYPYTFGGGTKVEIKSSADDAKKDAAKKDDAKKDDAKKDGEVQLVQSGAEVKKPGASVKVSCKASGYTFTDYNMDWVKQSPGQGLEWMGYIYPNNGGTGYNQKFKSKVTITVDTSTSTAYMELHSLRSEDTAVYYCATYGHYYGYMFAYWGQGTLVTVSSAAAFVPVFLPAKPTTTPAPRPPTPAPTIASQPLSLRPEACRPAAGGAVHTRGLDFACDIYIWAPLAGTCGVLLLSLVITLYCNHRNRSKRSRLLHSDYMNMTPRRPGPTRKHYQPYAPPRDFAAYRSRFSVVKRGRKKLLYIFKQPFMRPVQTTQEEDGCSCRFPEEEEGGCELRVKFSRSADAPAYQQGQNQLYNELNLGRREEYDVLDKRRGRDPEMGGKPRRKNPQEGLYNELQKDKMAEAYSEIGMKGERRRGKGHDGLYQGLSTATKDTYDALHMQALPPREFGSGVKQTLNFDLLKLAGDVESNPGPCMFHVSFRYIFGLPPLILVLLPVASSDCDIEGKDGKQYESVLMVSIDQLLDSMKEIGSNCLNNEFNFFKRHICDANKEGMFLFRAARKLRQFLKMNSTGDFDLHLLKVSEGTTILLNCTGQVKGRKPAALGEAQPTKSLEENKSLKEQKKLNDLCFLKRLLQEIKTCWNKILMGTKEHGSGVKQTLNFDLLKLAGDVESNPGPMALLLALSLLVLWTSPAPTLSGTNDAEDCCLSVTQKPIPGYIVRNFHYLLIKDGCRVPAVVFTTLRGRQLCAPPDQPWVERIIQRLQRTSAKMKRRSS

SEQ ID NO: 43 - DNA, 2625 bp, synthetic construct
  misc_feature 1..2625: note = anti-GM2 CAR (VH15VL)
  source 1..2625: mol_type = other DNA
atggactggacctggaggatcctcttcctggtggctgctgccacaggcgcccattccgaggtgcagctggtgcagtccggagccgaggtgaagaagcctggcgccagcgtgaaggtgagctgtaaggcctccggctacaccttcaccgactacaacatggactgggtcaagcagagccctggccagggcctggagtggatgggctatatctaccccaacaacggcggcaccggctacaaccagaagttcaagagcaaggtcaccatcaccgtggacacctccacctccacagcctacatggagctgcacagcctgaggagcgaggataccgccgtgtactactgcgctacctacggccattactacggatacatgttcgcctactggggccagggaaccctggtcaccgtgtcctccggaggaggaggaagcggaggcggcggctccggcggaggcggatccgacatccagctgacacaatcccccagcagcctgagcgctagccccggcgatagggtgacaattacctgcagcgcctccagctccgtgtcctacatgcactggtttcagcaaaagcccggcaaggcccctaagctgtggatctacagcaccagcaacctggccagcggagtgcctgccagatttagcggcagcggcagcggcaccagctacagcctgaccatcagcagactgcagcccgaggatatcgccacctactactgccagcagaggagctcctacccctacacattcggcggcggaaccaaggtggagatcaaggcggccgcattcgtgccggtcttcctgccagcgaagcccaccacgacgccagcgccgcgaccaccaacaccggcgcccaccatcgcgtcgcagcccctgtccctgcgcccagaggcgtgccggccagcggcggggggcgcagtgcacacgagggggctggacttcgcctgtgatatctacatctgggcgcccttggccgggacttgtggggtccttctcctgtcactggttatcaccctttactgcaaccacaggaacaggagtaagaggagcaggctcctgcacagtgactacatgaacatgactccccgccgccccgggcccacccgcaagcattaccagccctatgccccaccacgcgacttcgcagcctatcgctcccgtttctctgttgttaaacggggcagaaagaagctcctgtatatattcaaacaaccatttatgagaccagtacaaactactcaagaggaagatggctgtagctgccgatttccagaagaagaagaaggaggatgtgaactgagagtgaagttcagcaggagcgcagacgcccccgcgtaccagcagggccagaaccagctctataacgagctcaatctaggacgaagagaggagtacgatgttttggacaagagacgtggccgggaccctgagatggggggaaagccgagaaggaagaaccctcaggaaggcctgtacaatgaactgcagaaagataagatggcggaggcctacagtgagattgggatgaaaggcgagcgccggaggggcaaggggcacgatggcctttaccagggtctcagtacagccaccaaggacacctacgacgcccttcacatgcaggccctgccccctcgcgaattcggaagcggagtgaaacagactttgaattttgaccttctcaagttggcgggagacgtggagtccaaccctggaccatgcatgttccatgtttcttttaggtatatctttggacttcctcccctgatccttgttctgttgccagtagcatcatctgattgtgatattgaaggtaaagatggcaaacaatatgagagtgttctaatggtcagcatcgatcaattattggacagcatgaaagaaattggtagcaattgcctgaataatgaatttaacttttttaaaagacatatctgtgatgctaataaggaaggtatgtttttattccgtgctgctcgcaagttgaggcaatttcttaaaatgaatagcactggtgattttgatctccacttattaaaagtttcagaaggcacaacaatactgttgaactgcactggccaggttaaaggaagaaaaccagctgccctgggtgaagcccaaccaacaaagagtttggaagaaaataaatctttaaaggaacagaaaaaactgaatgacttgtgtttcctaaagagactattacaagagataaaaacttgttggaataaaattttgatgggcactaaagaacacggaagcggagtgaaacagactttgaattttgaccttctcaagttggcgggagacgtggagtccaaccctggacctatggccctgctactggccctcagcctgctggttctctggacttccccagccccaactctgagtggcaccaatgatgctgaagactgctgcctgtctgtgacccagaaacccatccctgggtacatcgtgaggaacttccactaccttctcatcaaggatggctgcagggtgcctgctgtagtgttcaccacactgaggggccgccagctctgtgcacccccagaccagccctgggtagaacgcatcatccagagactgcagaggacctcagccaagatgaagcgccgcagcagttaa

SEQ ID NO: 44 - protein, 874 aa, synthetic construct
  REGION 1..874: note = anti-GM2 CAR (VH15VL)
MDWTWRILFLVAAATGAHSEVQLVQSGAEVKKPGASVKVSCKASGYTFTDYNMDWVKQSPGQGLEWMGYIYPNNGGTGYNQKFKSKVTITVDTSTSTAYMELHSLRSEDTAVYYCATYGHYYGYMFAYWGQGTLVTVSSGGGGSGGGGSGGGGSDIQLTQSPSSLSASPGDRVTITCSASSSVSYMHWFQQKPGKAPKLWIYSTSNLASGVPARFSGSGSGTSYSLTISRLQPEDIATYYCQQRSSYPYTFGGGTKVEIKAAAFVPVFLPAKPTTTPAPRPPTPAPTIASQPLSLRPEACRPAAGGAVHTRGLDFACDIYIWAPLAGTCGVLLLSLVITLYCNHRNRSKRSRLLHSDYMNMTPRRPGPTRKHYQPYAPPRDFAAYRSRFSVVKRGRKKLLYIFKQPFMRPVQTTQEEDGCSCRFPEEEEGGCELRVKFSRSADAPAYQQGQNQLYNELNLGRREEYDVLDKRRGRDPEMGGKPRRKNPQEGLYNELQKDKMAEAYSEIGMKGERRRGKGHDGLYQGLSTATKDTYDALHMQALPPREFGSGVKQTLNFDLLKLAGDVESNPGPCMFHVSFRYIFGLPPLILVLLPVASSDCDIEGKDGKQYESVLMVSIDQLLDSMKEIGSNCLNNEFNFFKRHICDANKEGMFLFRAARKLRQFLKMNSTGDFDLHLLKVSEGTTILLNCTGQVKGRKPAALGEAQPTKSLEENKSLKEQKKLNDLCFLKRLLQEIKTCWNKILMGTKEHGSGVKQTLNFDLLKLAGDVESNPGPMALLLALSLLVLWTSPAPTLSGTNDAEDCCLSVTQKPIPGYIVRNFHYLLIKDGCRVPAVVFTTLRGRQLCAPPDQPWVERIIQRLQRTSAKMKRRSS

SEQ ID NO: 45 - DNA, 2655 bp, synthetic construct
  misc_feature 1..2655: note = anti-GM2 CAR (VH25VL)
  source 1..2655: mol_type = other DNA
atggactggacctggaggatcctgttcctggtggctgctgccaccggagcccactccgaagtgcagctggtgcagtccggagctgaggtgaagaagcccggcgccagcgtgaaggtcagctgcaaagccagcggctataccttcaccgactacaacatggactgggtgaagcagagccccggccaaggcctcgagtggatgggatacatctaccccaacaacggcggcaccggctacaaccagaagttcaagagcaaggtgaccatcaccgtggacacatccacaagcaccgcctatatggagctccacagcctgaggagcgaggacaccgccgtgtactactgcgccacctacggccactactacggctatatgttcgcctactggggccagggcaccctggtgacagtgtcctcctccagcgccgatgatgccaagaaggatgccgccaaaaaggacgacgctaagaaggatgacgccaagaaggacggcgatatccagctgacacagagccctagctccctgagcgctagccctggcgacagagtgaccatcacctgcagcgccagctccagcgtgagctacatgcactggttccagcagaaacccggcaaggcccccaagctgtggatctacagcaccagcaatctggctagcggcgtgcctgccaggtttagcggatccggcagcggcacctcctactccctgacaatctccagactgcagcccgaggacatcgccacctactactgccaacagaggtcctcctacccctacaccttcggcggcggcaccaaagtggagatcaaggcggccgcattcgtgccggtcttcctgccagcgaagcccaccacgacgccagcgccgcgaccaccaacaccggcgcccaccatcgcgtcgcagcccctgtccctgcgcccagaggcgtgccggccagcggcggggggcgcagtgcacacgagggggctggacttcgcctgtgatatctacatctgggcgcccttggccgggacttgtggggtccttctcctgtcactggttatcaccctttactgcaaccacaggaacaggagtaagaggagcaggctcctgcacagtgactacatgaacatgactccccgccgccccgggcccacccgcaagcattaccagccctatgccccaccacgcgacttcgcagcctatcgctcccgtttctctgttgttaaacggggcagaaagaagctcctgtatatattcaaacaaccatttatgagaccagtacaaactactcaagaggaagatggctgtagctgccgatttccagaagaagaagaaggaggatgtgaactgagagtgaagttcagcaggagcgcagacgcccccgcgtaccagcagggccagaaccagctctataacgagctcaatctaggacgaagagaggagtacgatgttttggacaagagacgtggccgggaccctgagatggggggaaagccgagaaggaagaaccctcaggaaggcctgtacaatgaactgcagaaagataagatggcggaggcctacagtgagattgggatgaaaggcgagcgccggaggggcaaggggcacgatggcctttaccagggtctcagtacagccaccaaggacacctacgacgcccttcacatgcaggccctgccccctcgcgaattcggaagcggagtgaaacagactttgaattttgaccttctcaagttggcgggagacgtggagtccaaccctggaccatgcatgttccatgtttcttttaggtatatctttggacttcctcccctgatccttgttctgttgccagtagcatcatctgattgtgatattgaaggtaaagatggcaaacaatatgagagtgttctaatggtcagcatcgatcaattattggacagcatgaaagaaattggtagcaattgcctgaataatgaatttaacttttttaaaagacatatctgtgatgctaataaggaaggtatgtttttattccgtgctgctcgcaagttgaggcaatttcttaaaatgaatagcactggtgattttgatctccacttattaaaagtttcagaaggcacaacaatactgttgaactgcactggccaggttaaaggaagaaaaccagctgccctgggtgaagcccaaccaacaaagagtttggaagaaaataaatctttaaaggaacagaaaaaactgaatgacttgtgtttcctaaagagactattacaagagataaaaacttgttggaataaaattttgatgggcactaaagaacacggaagcggagtgaaacagactttgaattttgaccttctcaagttggcgggagacgtggagtccaaccctggacctatggccctgctactggccctcagcctgctggttctctggacttccccagccccaactctgagtggcaccaatgatgctgaagactgctgcctgtctgtgacccagaaacccatccctgggtacatcgtgaggaacttccactaccttctcatcaaggatggctgcagggtgcctgctgtagtgttcaccacactgaggggccgccagctctgtgcacccccagaccagccctgggtagaacgcatcatccagagactgcagaggacctcagccaagatgaagcgccgcagcagttaa

SEQ ID NO: 46 - protein, 884 aa, synthetic construct
  REGION 1..884: note = anti-GM2 CAR (VH25VL)
MDWTWRILFLVAAATGAHSEVQLVQSGAEVKKPGASVKVSCKASGYTFTDYNMDWVKQSPGQGLEWMGYIYPNNGGTGYNQKFKSKVTITVDTSTSTAYMELHSLRSEDTAVYYCATYGHYYGYMFAYWGQGTLVTVSSSSADDAKKDAAKKDDAKKDDAKKDGDIQLTQSPSSLSASPGDRVTITCSASSSVSYMHWFQQKPGKAPKLWIYSTSNLASGVPARFSGSGSGTSYSLTISRLQPEDIATYYCQQRSSYPYTFGGGTKVEIKAAAFVPVFLPAKPTTTPAPRPPTPAPTIASQPLSLRPEACRPAAGGAVHTRGLDFACDIYIWAPLAGTCGVLLLSLVITLYCNHRNRSKRSRLLHSDYMNMTPRRPGPTRKHYQPYAPPRDFAAYRSRFSVVKRGRKKLLYIFKQPFMRPVQTTQEEDGCSCRFPEEEEGGCELRVKFSRSADAPAYQQGQNQLYNELNLGRREEYDVLDKRRGRDPEMGGKPRRKNPQEGLYNELQKDKMAEAYSEIGMKGERRRGKGHDGLYQGLSTATKDTYDALHMQALPPREFGSGVKQTLNFDLLKLAGDVESNPGPCMFHVSFRYIFGLPPLILVLLPVASSDCDIEGKDGKQYESVLMVSIDQLLDSMKEIGSNCLNNEFNFFKRHICDANKEGMFLFRAARKLRQFLKMNSTGDFDLHLLKVSEGTTILLNCTGQVKGRKPAALGEAQPTKSLEENKSLKEQKKLNDLCFLKRLLQEIKTCWNKILMGTKEHGSGVKQTLNFDLLKLAGDVESNPGPMALLLALSLLVLWTSPAPTLSGTNDAEDCCLSVTQKPIPGYIVRNFHYLLIKDGCRVPAVVFTTLRGRQLCAPPDQPWVERIIQRLQRTSAKMKRRSS

SEQ ID NO: 47 - DNA, 3825 bp, synthetic construct
  misc_feature 1..3825: note = anti-GM2 CAR (VL15VH)_HSV tk
  source 1..3825: mol_type = other DNA
atggattggacctggaggattctgttcctggtggctgctgccacaggcgcccattccgacatccagctgacccagtcccctagcagcctgtccgctagccccggagacagagtgaccatcacctgttccgccagctccagcgtgagctacatgcactggttccagcagaagcccggcaaggcccccaagctgtggatctacagcaccagcaacctggcttccggcgtgcctgccagattttccggctccggcagcggcacaagctactccctgaccatcagcagactgcagcccgaagacatcgccacctactactgtcagcagaggagcagctacccctacaccttcggcggcggcaccaaggtggagatcaagggcggcggcggaagcggaggcggcggcagcggcggaggcggaagcgaagtgcagctggtgcagtccggagccgaggtgaaaaagcctggcgcctccgtcaaggtgagctgcaaggccagcggctatacattcaccgactataacatggactgggtgaagcagagccccggccagggactggagtggatgggctacatctaccccaataacggcggcaccggctacaaccagaagttcaagtccaaggtgaccatcaccgtggacaccagcaccagcaccgcctacatggaactgcacagcctcagaagcgaagacaccgctgtgtactactgcgccacctacggccactactacggctacatgttcgcctactggggacagggcaccctggtgaccgtcagcagcgcggccgcattcgtgccggtcttcctgccagcgaagcccaccacgacgccagcgccgcgaccaccaacaccggcgcccaccatcgcgtcgcagcccctgtccctgcgcccagaggcgtgccggccagcggcggggggcgcagtgcacacgagggggctggacttcgcctgtgatatctacatctgggcgcccttggccgggacttgtggggtccttctcctgtcactggttatcaccctttactgcaaccacaggaacaggagtaagaggagcaggctcctgcacagtgactacatgaacatgactccccgccgccccgggcccacccgcaagcattaccagccctatgccccaccacgcgacttcgcagcctatcgctcccgtttctctgttgttaaacggggcagaaagaagctcctgtatatattcaaacaaccatttatgagaccagtacaaactactcaagaggaagatggctgtagctgccgatttccagaagaagaagaaggaggatgtgaactgagagtgaagttcagcaggagcgcagacgcccccgcgtaccagcagggccagaaccagctctataacgagctcaatctaggacgaagagaggagtacgatgttttggacaagagacgtggccgggaccctgagatggggggaaagccgagaaggaagaaccctcaggaaggcctgtacaatgaactgcagaaagataagatggcggaggcctacagtgagattgggatgaaaggcgagcgccggaggggcaaggggcacgatggcctttaccagggtctcagtacagccaccaaggacacctacgacgcccttcacatgcaggccctgccccctcgcgaattcggaagcggagtgaaacagactttgaattttgaccttctcaagttggcgggagacgtggagtccaaccctggaccatgcatgttccatgtgagcttcaggtacatcttcggactgcctcctctcatcctggtcctcctccccgtggccagctccgactgtgacatcgaaggaaaggatggcaagcagtacgaaagcgtgctgatggtgagcatcgatcagctcctggattccatgaaggaaatcggctccaactgcctcaacaatgagttcaacttttttaagaggcatatctgcgacgccaacaaggagggcatgtttctgttcagggccgccaggaagctgagacagttcctcaagatgaatagcaccggcgacttcgacctccatctgctgaaggtgtccgagggaaccaccatcctgctgaactgcaccggccaagtgaagggaagaaaacctgctgccctgggcgaggctcagcctaccaagagcctcgaggagaacaaaagcctgaaggagcagaagaagctgaacgacctgtgcttcctcaagaggctcctgcaggagattaagacctgttggaacaagatcctgatgggcacaaaggagcacggatccggcgtgaagcagaccctgaactttgacctgctcaaactggccggcgacgtcgagtccaatcctggacctatggctctgctgctcgccctgagcctgctcgtcctctggacctcccctgctcctaccctgagcggcaccaatgacgctgaagactgctgcctgtccgtgacccagaagcctatccccggatatatcgtgaggaattttcattacctcctgatcaaggacggctgtagagtgcccgccgtcgtgttcacaacactcagaggcaggcagctgtgtgctccccccgaccagccttgggtggagagaatcattcagagactgcaaaggacctccgctaagatgaagaggaggtccagcggcagcggagtgaagcagacactgaatttcgacctgctcaagctggccggcgatgtggagagcaaccctggacctatggcttcctaccccggacatcagcacgcttccgccttcgaccaggccgctagaagcagaggacactccaatagaaggacagccctgaggcctaggagacagcaggaggccaccgaggtgaggcccgagcagaaaatgcccaccctgctgagagtgtatattgatggaccccacggcatgggaaaaaccaccacaacccagctgctggtggctctgggaagcagggatgatattgtgtacgtccccgaacctatgacatattggagggtcctcggcgcctccgagaccatcgccaacatttacaccacccagcacaggctggatcagggagagatctccgccggcgatgctgccgtggtgatgaccagcgcccagatcactatgggtatgccttatgccgtgaccgacgctgtgctggctcctcacattggcggcgaagccggatcctcccatgctccccctcctgccctcacactgatctttgacagacatcctatcgccgctctgctgtgctaccccgccgctaggtacctgatgggcagcatgacccctcaggccgtgctggcttttgtggccctcattccccccacactgcctggcacaaatatcgtgctcggcgccctgcctgaggacaggcacatcgataggctggctaagagacagagacccggagagaggctggatctcgctatgctggccgccatcaggagggtgtacggcctgctggccaacaccgtgagatatctccagtgtggcggatcctggagggaagactggggccaactgagcggcacagctgtgcctcctcaaggcgctgagccccagagcaacgctggacccagacctcacatcggcgataccctgttcaccctgtttagagcccctgagctcctggcccctaacggcgacctgtacaatgtgttcgcttgggccctggatgtgctcgccaagagactcaggagcatgcacgtcttcattctggactacgaccagtcccccgctggctgcagagatgccctgctccagctgacctccggcatggtgcagacccacgtgaccacccctggaagcatccccacaatctgcgacctggccaggacctttgccagagaaatgggagaagccaac

SEQ ID NO: 48 - protein, 1275 aa, synthetic construct
  REGION 1..1275: note = anti-GM2 CAR (VL15VH)_HSV tk
MDWTWRILFLVAAATGAHSDIQLTQSPSSLSASPGDRVTITCSASSSVSYMHWFQQKPGKAPKLWIYSTSNLASGVPARFSGSGSGTSYSLTISRLQPEDIATYYCQQRSSYPYTFGGGTKVEIKGGGGSGGGGSGGGGSEVQLVQSGAEVKKPGASVKVSCKASGYTFTDYNMDWVKQSPGQGLEWMGYIYPNNGGTGYNQKFKSKVTITVDTSTSTAYMELHSLRSEDTAVYYCATYGHYYGYMFAYWGQGTLVTVSSAAAFVPVFLPAKPTTTPAPRPPTPAPTIASQPLSLRPEACRPAAGGAVHTRGLDFACDIYIWAPLAGTCGVLLLSLVITLYCNHRNRSKRSRLLHSDYMNMTPRRPGPTRKHYQPYAPPRDFAAYRSRFSVVKRGRKKLLYIFKQPFMRPVQTTQEEDGCSCRFPEEEEGGCELRVKFSRSADAPAYQQGQNQLYNELNLGRREEYDVLDKRRGRDPEMGGKPRRKNPQEGLYNELQKDKMAEAYSEIGMKGERRRGKGHDGLYQGLSTATKDTYDALHMQALPPREFGSGVKQTLNFDLLKLAGDVESNPGPCMFHVSFRYIFGLPPLILVLLPVASSDCDIEGKDGKQYESVLMVSIDQLLDSMKEIGSNCLNNEFNFFKRHICDANKEGMFLFRAARKLRQFLKMNSTGDFDLHLLKVSEGTTILLNCTGQVKGRKPAALGEAQPTKSLEENKSLKEQKKLNDLCFLKRLLQEIKTCWNKILMGTKEHGSGVKQTLNFDLLKLAGDVESNPGPMALLLALSLLVLWTSPAPTLSGTNDAEDCCLSVTQKPIPGYIVRNFHYLLIKDGCRVPAVVFTTLRGRQLCAPPDQPWVERIIQRLQRTSAKMKRRSSGSGVKQTLNFDLLKLAGDVESNPGPMASYPGHQHASAFDQAARSRGHSNRRTALRPRRQQEATEVRPEQKMPTLLRVYIDGPHGMGKTTTTQLLVALGSRDDIVYVPEPMTYWRVLGASETIANIYTTQHRLDQGEISAGDAAVVMTSAQITMGMPYAVTDAVLAPHIGGEAGSSHAPPPALTLIFDRHPIAALLCYPAARYLMGSMTPQAVLAFVALIPPTLPGTNIVLGALPEDRHIDRLAKRQRPGERLDLAMLAAIRRVYGLLANTVRYLQCGGSWREDWGQLSGTAVPPQGAEPQSNAGPRPHIGDTLFTLFRAPELLAPNGDLYNVFAWALDVLAKRLRSMHVFILDYDQSPAGCRDALLQLTSGMVQTHVTTPGSIPTICDLARTFAREMGEAN

SEQ ID NO: 49 - DNA, 360 bp, synthetic construct
  misc_feature 1..360: note = VH region of anti-GM2 antibody for VL25VH
  source 1..360: mol_type = other DNA
gaagtccagctggtgcagagcggcgctgaggtgaagaagcctggcgccagcgtcaaggtgagctgtaaggcctccggctacaccttcaccgactacaacatggattgggtgaagcagagccccggacagggcctggagtggatgggctacatctaccccaacaacggcggcaccggctacaaccagaaattcaagtccaaggtgaccatcaccgtggacaccagcacatccaccgcctacatggaactgcacagcctgaggtccgaggacacagccgtgtactactgcgctacctacggccactactacggctacatgttcgcttactggggacagggcaccctggtgaccgtgagctcc

SEQ ID NO: 50 - DNA, 318 bp, synthetic construct
  misc_feature 1..318: note = VL region of anti-GM2 antibody for VL25VH
  source 1..318: mol_type = other DNA
gatatccaactgacccagtccccttccagcctgagcgcttcccccggagacagggtgacaattacctgcagcgccagctcctccgtgagctacatgcactggttccagcagaagcccggcaaggcccccaagctgtggatctactccacaagcaacctggcctccggcgtgcctgccagatttagcggaagcggcagcggcacatcctacagcctgaccatctccaggctgcagcccgaggacatcgccacatactactgccagcagaggtccagctacccttacacattcggaggcggcaccaaggtggagatcaag

SEQ ID NO: 51 - DNA, 360 bp, synthetic construct
  misc_feature 1..360: note = VH region of anti-GM2 antibody for VH15VL
  source 1..360: mol_type = other DNA
gaggtgcagctggtgcagtccggagccgaggtgaagaagcctggcgccagcgtgaaggtgagctgtaaggcctccggctacaccttcaccgactacaacatggactgggtcaagcagagccctggccagggcctggagtggatgggctatatctaccccaacaacggcggcaccggctacaaccagaagttcaagagcaaggtcaccatcaccgtggacacctccacctccacagcctacatggagctgcacagcctgaggagcgaggataccgccgtgtactactgcgctacctacggccattactacggatacatgttcgcctactggggccagggaaccctggtcaccgtgtcctcc

SEQ ID NO: 52 - DNA, 318 bp, synthetic construct
  misc_feature 1..318: note = VL region of anti-GM2 antibody for VH15VL
  source 1..318: mol_type = other DNA
gacatccagctgacacaatcccccagcagcctgagcgctagccccggcgatagggtgacaattacctgcagcgcctccagctccgtgtcctacatgcactggtttcagcaaaagcccggcaaggcccctaagctgtggatctacagcaccagcaacctggccagcggagtgcctgccagatttagcggcagcggcagcggcaccagctacagcctgaccatcagcagactgcagcccgaggatatcgccacctactactgccagcagaggagctcctacccctacacattcggcggcggaaccaaggtggagatcaag

SEQ ID NO: 53 - DNA, 360 bp, synthetic construct
  misc_feature 1..360: note = VH region of anti-GM2 antibody for VH25VL
  source 1..360: mol_type = other DNA
gaagtgcagctggtgcagtccggagctgaggtgaagaagcccggcgccagcgtgaaggtcagctgcaaagccagcggctataccttcaccgactacaacatggactgggtgaagcagagccccggccaaggcctcgagtggatgggatacatctaccccaacaacggcggcaccggctacaaccagaagttcaagagcaaggtgaccatcaccgtggacacatccacaagcaccgcctatatggagctccacagcctgaggagcgaggacaccgccgtgtactactgcgccacctacggccactactacggctatatgttcgcctactggggccagggcaccctggtgacagtgtcctcc

SEQ ID NO: 54 - DNA, 318 bp, synthetic construct
  misc_feature 1..318: note = VL region of anti-GM2 antibody for VH25VL
  source 1..318: mol_type = other DNA
gatatccagctgacacagagccctagctccctgagcgctagccctggcgacagagtgaccatcacctgcagcgccagctccagcgtgagctacatgcactggttccagcagaaacccggcaaggcccccaagctgtggatctacagcaccagcaatctggctagcggcgtgcctgccaggtttagcggatccggcagcggcacctcctactccctgacaatctccagactgcagcccgaggacatcgccacctactactgccaacagaggtcctcctacccctacaccttcggcggcggcaccaaagtggagatcaag

SEQ ID NO: 55 - DNA, 45 bp, synthetic construct
  misc_feature 1..45: note = linker 15 for VH15VL
  source 1..45: mol_type = other DNA
ggaggaggaggaagcggaggcggcggctccggcggaggcggatcc

SEQ ID NO: 56 - DNA, 75 bp, synthetic construct
  misc_feature 1..75: note = linker 25 for VH25VL
  source 1..75: mol_type = other DNA
tccagcgccgatgatgccaagaaggatgccgccaaaaaggacgacgctaagaaggatgacgccaagaaggacggc

SEQ ID NO: 57 - protein, 19 aa, synthetic construct
  REGION 1..19: note = signal peptide
MDWTWRILFLVAAATGAHS

SEQ ID NO: 58 - DNA, 531 bp, Homo sapiens
  source 1..531: mol_type = other DNA
atgttccatgtttcttttaggtatatctttggacttcctcccctgatccttgttctgttgccagtagcatcatctgattgtgatattgaaggtaaagatggcaaacaatatgagagtgttctaatggtcagcatcgatcaattattggacagcatgaaagaaattggtagcaattgcctgaataatgaatttaacttttttaaaagacatatctgtgatgctaataaggaaggtatgtttttattccgtgctgctcgcaagttgaggcaatttcttaaaatgaatagcactggtgattttgatctccacttattaaaagtttcagaaggcacaacaatactgttgaactgcactggccaggttaaaggaagaaaaccagctgccctgggtgaagcccaaccaacaaagagtttggaagaaaataaatctttaaaggaacagaaaaaactgaatgacttgtgtttcctaaagagactattacaagagataaaaacttgttggaataaaattttgatgggcactaaagaacac

SEQ ID NO: 59 - protein, 177 aa, Homo sapiens
MFHVSFRYIFGLPPLILVLLPVASSDCDIEGKDGKQYESVLMVSIDQLLDSMKEIGSNCLNNEFNFFKRHICDANKEGMFLFRAARKLRQFLKMNSTGDFDLHLLKVSEGTTILLNCTGQVKGRKPAALGEAQPTKSLEENKSLKEQKKLNDLCFLKRLLQEIKTCWNKILMGTKEH

SEQ ID NO: 60 - DNA, 294 bp, Homo sapiens
  source 1..294: mol_type = other DNA
atggccctgctactggccctcagcctgctggttctctggacttccccagccccaactctgagtggcaccaatgatgctgaagactgctgcctgtctgtgacccagaaacccatccctgggtacatcgtgaggaacttccactaccttctcatcaaggatggctgcagggtgcctgctgtagtgttcaccacactgaggggccgccagctctgtgcacccccagaccagccctgggtagaacgcatcatccagagactgcagaggacctcagccaagatgaagcgccgcagcagt

SEQ ID NO: 61 - protein, 98 aa, Homo sapiens
MALLLALSLLVLWTSPAPTLSGTNDAEDCCLSVTQKPIPGYIVRNFHYLLIKDGCRVPAVVFTTLRGRQLCAPPDQPWVERIIQRLQRTSAKMKRRSS

SEQ ID NO: 62 - protein, 25 aa, synthetic construct
  REGION 1..25: note = F2A
GSGVKQTLNFDLLKLAGDVESNPGP

SEQ ID NO: 63 - protein, 5 aa, synthetic construct
  REGION 1..5: note = CDR1 of VH region of anti-GM2 antibody
DYNMD

SEQ ID NO: 64 - protein, 17 aa, synthetic construct
  REGION 1..17: note = CDR2 of VH region of anti-GM2 antibody
YIYPNNGGTGYNQKFKS

SEQ ID NO: 65 - protein, 11 aa, synthetic construct
  REGION 1..11: note = CDR3 of VH region of anti-GM2 antibody
YGHYYGYMFAY

SEQ ID NO: 66 - protein, 10 aa, synthetic construct
  REGION 1..10: note = CDR1 of VL region of anti-GM2 antibody
SASSSVSYMH

SEQ ID NO: 67 - protein, 7 aa, synthetic construct
  REGION 1..7: note = CDR2 of VL region of anti-GM2 antibody
STSNLAS

SEQ ID NO: 68 - protein, 9 aa, synthetic construct
  REGION 1..9: note = CDR3 of VL region of anti-GM2 antibody
QQRSSYPYT